European Patent Application EP 4 707 397 A1, published March 11, 2026. Title: Promoter for Expression of a Gene in Retinal Cell and Vector System Comprising the Same. Applicant: 한국생명공학연구원. Application KR. The sequence listing filed with the application follows.

SEQUENCE LISTING (41 sequences)

SEQ ID NO: 1 - DNA, 482 bp, synthetic construct
  source 1..482: mol_type = other DNA
ggcccaggcttcccagcagggctaaggatatgcaaggagtgcattcatccggaggtgttggcagcatcccagccccaccccattctcatcgtaaatcaggctcacttccattggctgcatacggtggagtgatgtgaccatatgtcacttgagcattacacaaatcctaatgagctaaaaatatgtttgttttagctaattgacctctttggccttcataaagcagttggtaaacatcctcagataatgatttccaaagaggtcgacgggccccagaagcctggtggttgtttgtccttctcaggggaaaagtgaggcggccccttggaggaaggggccgggcagaatgatctaatcggattccaagcagctcaggggattgtctttttctagcaccttcttgccactcctaagcgtcctccgtgaccccggctgggatttagcctggtgctgtgtcagccccgggctcccaggggcttccc

SEQ ID NO: 2 - DNA, 650 bp, synthetic construct
  source 1..650: mol_type = other DNA
ggcccaggcttcccagcagggctaaggatatgcaaggagtgcattcatccggaggtgttggcagcatcccagccccaccccattctcatcgtaaatcaggctcacttccattggctgcatacggtggagtgatgtgaccatatgtcacttgagcattacacaaatcctaatgagctaaaaatatgtttgttttagctaattgacctctttggccttcataaagcagttggtaaacatcctcagataatgatttccaaagaggtcgacgggccccagaagcctggtggttgtttgtccttctcaggggaaaagtgaggcggccccttggaggaaggggccgggcagaatgatctaatcggattccaagcagctcaggggattgtctttttctagcaccttcttgccactcctaagcgtcctccgtgaccccggctgggatttagcctggtgctgtgtcagccccgggctcccaggggcttcccagtggtccccaggaaccctcgacagggccagggcgtctctctcgtccagcaagggcagggacgggccacaggccaagggcagcagtcaggcctgctctgtctgtgaacgctcccggcttggcctcggctgatgggccctcacgcctgaagcgggcaggaagctccggg

SEQ ID NO: 3 - DNA, 381 bp, synthetic construct
  source 1..381: mol_type = other DNA
ggcccaggcttcccagcagggctaaggatatgcaaggagtgcattcatccggaggtgttggcagcatcccagccccaccccattctcatcgtaaatcaggctcacttccattggctgcatacggtggagtgatgtgaccatatgtcacttgagcattacacaaatcctaatgagctaaaaatatgtttgttttagctaattgacctctttggccttcataaagcagttggtaaacatcctcagataatgatttccaaagaggtcgacgtcccagggtctgaggagagggagcgcaggcccccatttgtaggagtgagtcagctgacccgcccccggggttcctaatctcactaagaaagactttgctgatgacagggtttc

SEQ ID NO: 4 - DNA, 435 bp, synthetic construct
  source 1..435: mol_type = other DNA
ggcccaggcttcccagcagggctaaggatatgcaaggagtgcattcatccggaggtgttggcagcatcccagccccaccccattctcatcgtaaatcaggctcacttccattggctgcatacggtggagtgatgtgaccatatgtcacttgagcattacacaaatcctaatgagctaaaaatatgtttgttttagctaattgacctctttggccttcataaagcagttggtaaacatcctcagataatgatttccaaagaggtcgacgtcccagggtctgaggagagggagcgcaggcccccatttgtaggagtgagtcagctgacccgcccccggggttcctaatctcactaagaaagactttgctgatgacagggtttcctgggagtccatgcgtgcctggagcagcagcgtctccagggacaggcagccacc

SEQ ID NO: 5 - DNA, 261 bp, synthetic construct
  source 1..261: mol_type = other DNA
ggcccaggcttcccagcagggctaaggatatgcaaggagtgcattcatccggaggtgttggcagcatcccagccccaccccattctcatcgtaaatcaggctcacttccattggctgcatacggtggagtgatgtgaccatatgtcacttgagcattacacaaatcctaatgagctaaaaatatgtttgttttagctaattgacctctttggccttcataaagcagttggtaaacatcctcagataatgatttccaaagag

SEQ ID NO: 6 - DNA, 215 bp, synthetic construct
  source 1..215: mol_type = other DNA
gggccccagaagcctggtggttgtttgtccttctcaggggaaaagtgaggcggccccttggaggaaggggccgggcagaatgatctaatcggattccaagcagctcaggggattgtctttttctagcaccttcttgccactcctaagcgtcctccgtgaccccggctgggatttagcctggtgctgtgtcagccccgggctcccaggggcttccc

SEQ ID NO: 7 - DNA, 114 bp, synthetic construct
  source 1..114: mol_type = other DNA
gtcccagggtctgaggagagggagcgcaggcccccatttgtaggagtgagtcagctgacccgcccccggggttcctaatctcactaagaaagactttgctgatgacagggtttc

SEQ ID NO: 8 - DNA, 168 bp, synthetic construct
  source 1..168: mol_type = other DNA
agtggtccccaggaaccctcgacagggccagggcgtctctctcgtccagcaagggcagggacgggccacaggccaagggcagcagtcaggcctgctctgtctgtgaacgctcccggcttggcctcggctgatgggccctcacgcctgaagcgggcaggaagctccggg

SEQ ID NO: 9 - DNA, 54 bp, synthetic construct
  source 1..54: mol_type = other DNA
ctgggagtccatgcgtgcctggagcagcagcgtctccagggacaggcagccacc

SEQ ID NO: 10 - DNA, 544 bp, synthetic construct
  source 1..544: mol_type = other DNA
tccaggggcgtgcacagggcggggccggtcatgcgcggtcctagtttgagttcaggggcgggatccaggggcgtgcacagggcggggccgctcatgcgcggccctagtttgagttcaggggcgggatccaggggcgtgcacagggcggggaagaggtcgacgggccccagaagcctggtggttgtttgtccttctcaggggaaaagtgaggcggccccttggaggaaggggccgggcagaatgatctaatcggattccaagcagctcaggggattgtctttttctagcaccttcttgccactcctaagcgtcctccgtgaccccggctgggatttagcctggtgctgtgtcagccccgggctcccaggggcttcccagtggtccccaggaaccctcgacagggccagggcgtctctctcgtccagcaagggcagggacgggccacaggccaagggcagcagtcaggcctgctctgtctgtgaacgctcccggcttggcctcggctgatgggccctcacgcctgaagcgggcaggaagctccggg

SEQ ID NO: 11 - DNA, 329 bp, synthetic construct
  source 1..329: mol_type = other DNA
tccaggggcgtgcacagggcggggccggtcatgcgcggtcctagtttgagttcaggggcgggatccaggggcgtgcacagggcggggccgctcatgcgcggccctagtttgagttcaggggcgggatccaggggcgtgcacagggcggggaagaggtcgacgtcccagggtctgaggagagggagcgcaggcccccatttgtaggagtgagtcagctgacccgcccccggggttcctaatctcactaagaaagactttgctgatgacagggtttcctgggagtccatgcgtgcctggagcagcagcgtctccagggacaggcagccacc

SEQ ID NO: 12 - DNA, 150 bp, synthetic construct
  source 1..150: mol_type = other DNA
tccaggggcgtgcacagggcggggccggtcatgcgcggtcctagtttgagttcaggggcgggatccaggggcgtgcacagggcggggccgctcatgcgcggccctagtttgagttcaggggcgggatccaggggcgtgcacagggcgggg

SEQ ID NO: 13 - DNA, 63 bp, synthetic construct
  source 1..63: mol_type = other DNA
tccaggggcgtgcacagggcggggccggtcatgcgcggtcctagtttgagttcaggggcggga

SEQ ID NO: 14 - DNA, 56 bp, synthetic construct
  source 1..56: mol_type = other DNA
gcgtgcacagggcggggccggtcatgcgcggtcctagtttgagttcaggggcggga

SEQ ID NO: 15 - DNA, 50 bp, synthetic construct
  source 1..50: mol_type = other DNA
tccaggggcgtgcacagggcggggccggtcatgcgcggtcctagtttgag

SEQ ID NO: 16 - DNA, 43 bp, synthetic construct
  source 1..43: mol_type = other DNA
ggggccggtcatgcgcggtcctagtttgagttcaggggcggga

SEQ ID NO: 17 - DNA, 42 bp, synthetic construct
  source 1..42: mol_type = other DNA
tccaggggcgtgcacagggcggggccggtcatgcgcggtcct

SEQ ID NO: 18 - DNA, 35 bp, synthetic construct
  source 1..35: mol_type = other DNA
gcgtgcacagggcggggccggtcatgcgcggtcct

SEQ ID NO: 19 - DNA, 1426 bp, synthetic construct
  source 1..1426: mol_type = other DNA
accaccaaatttagcattttcctgagtgaataggtgtgcacatgatgcctagttgctttcaaagaggggaatccatgacattttcatacaattcgagaatgttagtgcttatgtggcaggaaattgttcaaggtcaccccctaaaaaatgatggcgaagaaaggacgaaaacctgagacttctggttgtagttctctccctccattgcttcccttacattaagatagaatgaacagtatggtcgacggcccaggcttcccagcagggctaaggatatgcaaggagtgcattcatccggaggtgttggcagcatcccagccccaccccattctcatcgtaaatcaggctcacttccattggctgcatacggtggagtgatgtgaccatatgtcacttgagcattacacaaatcctaatgagctaaaaatatgtttgttttagctaattgacctctttggccttcataaagcagttggtaaacatcctcagataatgatttccaaagaggtcgaccgaaaagtatcttcctcgcgaactgaatctcagttgatgctagtatcttccatgagacttccttgttgaggcaggtaactctgtgggttaacttgatggggctcagccaaagacctaagaactaaatggattaagatgcttaatgaggccagggctcaacttaatcccctgctcctgggccagctctccagttcagtaaggtagagctttggccgaggacgaggggaagatgggagtcaaagttctgtttgccctgatctgcatcgctgtggccgaggccaagcccaccgagaacaacgaagacttcaacatcgtggccgtggccagcaacttcgcgaccacggatctcgatgctgaccgcgggaagttgcccggcaagaagctgccgctggaggtgctcaaagagctggaagccaatgcccggaaagctggctgcaccaggggctgtctgatctgcctgtcccacatcaagtgcacgcccaagatgaagaagttcatcccaggacgctgccacacctacgaaggcgacaaagagtccgcacagggcggcataggcgaggcgatcgtcgacattcctgagattcctgggttcaaggacttggagcccctggagcagttcatcgcacaggtcgatctgtgtgtggactgcacaactggctgcctcaaagggcttgccaacgtgcagtgttctgacctgctcaagaagtggctgccgcaacgctgtgcgacctttgccagcaagatccagggccaggtggacaagatcaagggggccggtggtgactaagcggccgctcgagcatgcatctagaaataattcttactgtcatgccaagtaagatgcttttctgtgctgcaatagcaggcatgctggggatgcggtgggctctatggcttctgaggcggaaagaac

SEQ ID NO: 20 - DNA, 768 bp, synthetic construct
  source 1..768: mol_type = other DNA
accaccaaatttagcattttcctgagtgaataggtgtgcacatgatgcctagttgctttcaaagaggggaatccatgacattttcatacaattcgagaatgttagtgcttatgtggcaggaaattgttcaaggtcaccccctaaaaaatgatggcgaagaaaggacgaaaacctgagacttctggttgtagttctctccctccattgcttcccttacattaagatagaatgaacagtatggtcgacggcccaggcttcccagcagggctaaggatatgcaaggagtgcattcatccggaggtgttggcagcatcccagccccaccccattctcatcgtaaatcaggctcacttccattggctgcatacggtggagtgatgtgaccatatgtcacttgagcattacacaaatcctaatgagctaaaaatatgtttgttttagctaattgacctctttggccttcataaagcagttggtaaacatcctcagataatgatttccaaagaggtcgacgggccccagaagcctggtggttgtttgtccttctcaggggaaaagtgaggcggccccttggaggaaggggccgggcagaatgatctaatcggattccaagcagctcaggggattgtctttttctagcaccttcttgccactcctaagcgtcctccgtgaccccggctgggatttagcctggtgctgtgtcagccccgggctcccaggggcttcccagttcagtaaggtagagctttggccgaggacgaggggaag

SEQ ID NO: 21 - DNA, 667 bp, synthetic construct
  source 1..667: mol_type = other DNA
accaccaaatttagcattttcctgagtgaataggtgtgcacatgatgcctagttgctttcaaagaggggaatccatgacattttcatacaattcgagaatgttagtgcttatgtggcaggaaattgttcaaggtcaccccctaaaaaatgatggcgaagaaaggacgaaaacctgagacttctggttgtagttctctccctccattgcttcccttacattaagatagaatgaacagtatggtcgacggcccaggcttcccagcagggctaaggatatgcaaggagtgcattcatccggaggtgttggcagcatcccagccccaccccattctcatcgtaaatcaggctcacttccattggctgcatacggtggagtgatgtgaccatatgtcacttgagcattacacaaatcctaatgagctaaaaatatgtttgttttagctaattgacctctttggccttcataaagcagttggtaaacatcctcagataatgatttccaaagaggtcgacgtcccagggtctgaggagagggagcgcaggcccccatttgtaggagtgagtcagctgacccgcccccggggttcctaatctcactaagaaagactttgctgatgacagggtttcagttcagtaaggtagagctttggccgaggacgaggggaag

SEQ ID NO: 22 - DNA, 240 bp, synthetic construct
  source 1..240: mol_type = other DNA
accaccaaatttagcattttcctgagtgaataggtgtgcacatgatgcctagttgctttcaaagaggggaatccatgacattttcatacaattcgagaatgttagtgcttatgtggcaggaaattgttcaaggtcaccccctaaaaaatgatggcgaagaaaggacgaaaacctgagacttctggttgtagttctctccctccattgcttcccttacattaagatagaatgaacagtatg

SEQ ID NO: 23 - DNA, 189 bp, synthetic construct
  source 1..189: mol_type = other DNA
cgaaaagtatcttcctcgcgaactgaatctcagttgatgctagtatcttccatgagacttccttgttgaggcaggtaactctgtgggttaacttgatggggctcagccaaagacctaagaactaaatggattaagatgcttaatgaggccagggctcaacttaatcccctgctcctgggccagctctcc

SEQ ID NO: 24 - DNA, 40 bp, synthetic construct
  source 1..40: mol_type = other DNA
agttcagtaaggtagagctttggccgaggacgaggggaag

SEQ ID NO: 25 - skipped

SEQ ID NO: 26 - DNA, 496 bp, synthetic construct
  source 1..496: mol_type = other DNA
ggcccaggcttcccagcagggctaaggatatgcaaggagtgcattcatccggaggtgttggcagcatcccagccccaccccattctcatcgtaaatcaggctcacttccattggctgcatacggtggagtgatgtgaccatatgtcacttgagcattacacaaatcctaatgagctaaaaatatgtttgttttagctaattgacctctttggccttcataaagcagttggtaaacatcctcagataatgatttccaaagaggtcgaccgaaaagtatcttcctcgcgaactgaatctcagttgatgctagtatcttccatgagacttccttgttgaggcaggtaactctgtgggttaacttgatggggctcagccaaagacctaagaactaaatggattaagatgcttaatgaggccagggctcaacttaatcccctgctcctgggccagctctccagttcagtaaggtagagctttggccgaggacgaggggaag

SEQ ID NO: 27 - DNA, 999 bp, synthetic construct
  source 1..999: mol_type = other DNA
tccaggggcgtgcacagggcggggccggtcatgcgcggtcctagtttgagttcaggggcgggatccaggggcgtgcacagggcggggccgctcatgcgcggccctagtttgagttcaggggcgggatccaggggcgtgcacagggcggggaagaggtcgacgtcccagggtctgaggagagggagcgcaggcccccatttgtaggagtgagtcagctgacccgcccccggggttcctaatctcactaagaaagactttgctgatgacagggtttcagttcagtaaggtagagctttggccgaggacgaggggaagatgggagtcaaagttctgtttgccctgatctgcatcgctgtggccgaggccaagcccaccgagaacaacgaagacttcaacatcgtggccgtggccagcaacttcgcgaccacggatctcgatgctgaccgcgggaagttgcccggcaagaagctgccgctggaggtgctcaaagagctggaagccaatgcccggaaagctggctgcaccaggggctgtctgatctgcctgtcccacatcaagtgcacgcccaagatgaagaagttcatcccaggacgctgccacacctacgaaggcgacaaagagtccgcacagggcggcataggcgaggcgatcgtcgacattcctgagattcctgggttcaaggacttggagcccctggagcagttcatcgcacaggtcgatctgtgtgtggactgcacaactggctgcctcaaagggcttgccaacgtgcagtgttctgacctgctcaagaagtggctgccgcaacgctgtgcgacctttgccagcaagatccagggccaggtggacaagatcaagggggccggtggtgactaagcggccgctcgagcatgcatctagaaataattcttactgtcatgccaagtaagatgcttttctgtgctgcaatagcaggcatgctggggatgcggtgggctctatggcttctgaggcggaaagaac

SEQ ID NO: 28 - DNA, 39 bp, synthetic construct
  source 1..39: mol_type = other DNA
tccaggggcgtgcacagggcggggccggtcatgcgcggt

SEQ ID NO: 29 - DNA, 24 bp, synthetic construct
  source 1..24: mol_type = other DNA
tccaggggcgtgcacagggcgggg

SEQ ID NO: 30 - DNA, 78 bp, synthetic construct
  source 1..78: mol_type = other DNA
tccaggggcgtgcacagggcggggccggtcatgcgcggttccaggggcgtgcacagggcggggccggtcatgcgcggt

SEQ ID NO: 31 - DNA, 48 bp, synthetic construct
  source 1..48: mol_type = other DNA
tccaggggcgtgcacagggcggggtccaggggcgtgcacagggcgggg

SEQ ID NO: 32 - DNA, 927 bp, synthetic construct
  source 1..927: mol_type = other DNA
tccaggggcgtgcacagggcggggccggtcatgcgcggttccaggggcgtgcacagggcggggccggtcatgcgcggtaagaggtcgacgtcccagggtctgaggagagggagcgcaggcccccatttgtaggagtgagtcagctgacccgcccccggggttcctaatctcactaagaaagactttgctgatgacagggtttcagttcagtaaggtagagctttggccgaggacgaggggaagatgggagtcaaagttctgtttgccctgatctgcatcgctgtggccgaggccaagcccaccgagaacaacgaagacttcaacatcgtggccgtggccagcaacttcgcgaccacggatctcgatgctgaccgcgggaagttgcccggcaagaagctgccgctggaggtgctcaaagagctggaagccaatgcccggaaagctggctgcaccaggggctgtctgatctgcctgtcccacatcaagtgcacgcccaagatgaagaagttcatcccaggacgctgccacacctacgaaggcgacaaagagtccgcacagggcggcataggcgaggcgatcgtcgacattcctgagattcctgggttcaaggacttggagcccctggagcagttcatcgcacaggtcgatctgtgtgtggactgcacaactggctgcctcaaagggcttgccaacgtgcagtgttctgacctgctcaagaagtggctgccgcaacgctgtgcgacctttgccagcaagatccagggccaggtggacaagatcaagggggccggtggtgactaagcggccgctcgagcatgcatctagaaataattcttactgtcatgccaagtaagatgcttttctgtgctgcaatagcaggcatgctggggatgcggtgggctctatggcttctgaggcggaaagaac

SEQ ID NO: 33 - DNA, 213 bp, synthetic construct
  source 1..213: mol_type = other DNA
tccaggggcgtgcacagggcggggtccaggggcgtgcacagggcggggaagaggtcgacgtcccagggtctgaggagagggagcgcaggcccccatttgtaggagtgagtcagctgacccgcccccggggttcctaatctcactaagaaagactttgctgatgacagggtttcagttcagtaaggtagagctttggccgaggacgaggggaag

SEQ ID NO: 34 - DNA, 11 bp, synthetic construct
  source 1..11: mol_type = other DNA
aagaggtcgac

SEQ ID NO: 35 - DNA, 57 bp, synthetic construct
  source 1..57: mol_type = other DNA
caatagcaggcatgctggggatgcggtgggctctatggcttctgaggcggaaagaac

SEQ ID NO: 36 - DNA, 225 bp, synthetic construct
  source 1..225: mol_type = other DNA
ctgtgccttctagttgccagccatctgttgtttgcccctcccccgtgccttccttgaccctggaaggtgccactcccactgtcctttcctaataaaatgaggaaattgcatcgcattgtctgagtaggtgtcattctattctggggggtggggtggggcaggacagcaagggggaggattgggaagacaatagcaggcatgctggggatgcggtgggctctatgg

SEQ ID NO: 37 - DNA, 20 bp, synthetic construct
  source 1..20: mol_type = other DNA
cactacgacgctgaggtcaa

SEQ ID NO: 38 - DNA, 20 bp, synthetic construct
  source 1..20: mol_type = other DNA
tagtcctcgttgtgggaggt

SEQ ID NO: 39 - DNA, 8061 bp, synthetic construct
  source 1..8061: mol_type = other DNA
gtaagggtctgagcgcagctggggaggctccgtgcatgggttacgtccctgtgtacatgtgtgtgcctgtgtgcacttgcacatacatgtgagtttgtgtatataggtgtgtctgtgtgcacatgggcgtctgtgtggttgtgcatttgtgtgcatgtgagtgttgtgaaccctgatatctgaggcaggtaccagttaatttagaaagtttattttgctgaggttgaggacgcgagtccgtggcagcctcaggaggtcctgatgacaggtggtcgccgcacagtttggttttacacattttagggagccatgagacatcaatcagcatatgtaagatgaacactggttcggtctggaaaggcgggagggggcttccaggtcataggaagatgagagacaaatggttacattcttttgagtttctgatgagtctctccagaggaggcaatcagataagcatttatctcagtgaacagagggctcactgagaggactttgaatacaatgggaggcaggtttgccataagcagttcccagcttgactctttcctttagtgattttgggtctcaagatattttccttttacagtgtgcctgtgtgcatgcctgtgtctctgtgcacacacgtgtgtctgtgtgcctgcatgtgtgcctgtgtgcccatgcctgtgtctctgtgcacacgtgtctgtgtgcctgtgtgtgcatgcccgtgtctgtgcacacacgtgtccgtgtacctgtatgtgcatgcctgcatctttgtgcacacatgtgtatccgtgtgcctgtgtctgtgtgcatgtgttcctgtgtatgcatgcccgggtctctgtgcacacgtgtgtccgtgtgcctgtatgtgagtgcacatgcacggtgcatcctactgcctcccccatcccgtgtcactcatctcctctcacctccccccaggcagggaggctcgcagcacctgtggaggagaggagacccccacagtcaagcagagcggggtccgtgttctgggcccagcacctgctggcgtgtggcctgtgtgctttacttaacctccgagcctcctgctagcactcggtgcacaggcttgctgaggagacctcacacgccacgtgcccggcgcctgtgtacagcagccacaccgtgaatttgagttcttcctctctcctccgcagtcttgagggtccgcgtgtcgggctcacttctgctgggatttccagagaatgtcgcttccccgtggttgttttggctgtggggaggcagtgctgtcgcctgatggggtttgtgtgcggtggtgttttgggtcctcccatgctggtgtttaggcactgggcgtatttgtgccgtggccacgggggggacatcctcgctccagctggacttaggggaaggtgcatctcggggtgggggctaaggactgtttccccaaagttctgacgaagggcagttctgtgcccacacccctcatggctgggttgccatctggatgtgggattccgtagccactgagtgctcagggccagtggtcgaaggtctcaaaactttctggaaggcagctcatcctgggggatcccatggctcaaggaagcctcgggtggcacctgcttttcgtgagatgatccaagcctctttctgggtgggtagaaacggttggcgctgcggccctcgagtctttgggacccttgccaagcctgggtgtgagcgcgtgggtggaagccccctcacgcatttcggggagatccaggtggactccgaggccaggactggaagagttaacctcacggatggaaagggcccagcttccaggccgagggtgagggcccgactggccgccagggggccccaagccttcgccggcgcccgttcctcggagccccaggtgctcacagcagggctgggctcaggctgtgacccctgcacagtgacctggagatgctgccgtcagggtgcaggctgggaggccggtgtcagttcagcaaagccgcagggtccgcatccttcttcctggcaccctcgcgccctcccacgcgccccccacgcagcgagagacaccacagccataagaagcctgtcgggggactcccccttgccagtgcggtgcggacccaggggcgtgcacagggcggggccggtcatgcgcggtcctagtttgaggtcaggggcgggatccaggggcgtgcacagggcggggccggtcatgcgcggtcctagtttgagttcaggggcgggatccaggggcgtgcacagggcggggccggtcatgcgcggccctagtttgaggtcaggggcgggatccaggggcgtgcacagggcggggccggtcatgcgcggtcctagtttgagttcaggggcgggatccaggggcgtgcacagggcggggccgctcatgcgcggccctagtttgagttcaggggcgggatccaggggcgtgcacagggcggggccggtcatgcgcggtcctagtttgagttcaggggcgggatccaggggcgtgcacagggcggggccggtcatgcgcggccctagtttgaggtcaggggcgggatccaggggcgtgcacagggcggggccggtcatgcgcggtcctagtttgagttcaggggcgggatccaggggcgtgcacagggcggggccggtcatgcgcggccctagtttgaggtcaggggcgggatccaggggcgtgcacagggcggggccggtcatgcgcggtcctagtttgaggtcaggggcgggacccaggggcgtgcacagggcggggccggtcatgcgcggtcctagtttgaggtcaggggcgggatccaggggcgtgcacagggcggggccggttatgcgcggtcctagtttgaggtcaggggcgggatccaggggcgtgcacagggcggggccggttatgcgcggtcctagtttgaggtcaggggcgggatccaggggcgtgcacagggcggggccggtcatgcgcggtcgtagtttgaggtcaggggcgggatccaggggcgtgcacagggcggggccggtcatgcgcggtcgtagtttgaggtcaggggcgggatccaggggcgtgcacagggcggggccggtcatgcgcggccctagtttgaggtcaggggcgggatccaggggcgtgcacagggcggggccggtcatgcgcggccctagtttgaggtcaggggcgggatccaggggcgtgcacagggcggggccggtcatgcgcggccctagtttgaggtcaggggcgggatccaggggcgtgcacagggcggggccggtcatgcgcggccctagtttgaggtcaggggcgggatccaggggcgtgcacagggcggggccggtcatgcgcggtcctagtttgagttcaggggcgggagaatttgtgaacagagcaggtagagctgtctccctcacgctttctgtcaatatttactggccgctgcgtggctgcaggtccctcaggaggcctggggcacaaacaggtgcgccgtccgggctgcatcatgggggtcaggccaggagggctgggggctccttggcccaggaactgacaggagcctgcggtctggtgggccttgctcgtgcccggcctgggagctgagaaggctctgggtgggtctagaggctgtgatcgtgtgagcagttcctccccggagtctgggcagaattctgacgtccgtgtaatcctggaccagtagggcatattcagggcctgtggttctgtgaggcagggttcctgcaactcttttggggaaaaaggattctgtggccacatcagcctggccctcaggcacggtgaaggaccaggaaggaccttgactcagaagtgtcaaaactgaccagccccagcagcccccatgccccagcctgcggcctctctgcctggtcccaggacatccgtcatgggtctcccaacgggcctgtccgccactgtgtgccgggttggcctcacttgggtagcagctggcaagttgacataactcacacaggccccatgtgccacacagagctggctcgggggccaggcaggtgtctgaacttctcctggagtctgactcaccagagcagacgtctgccaaggaccctgcttggtcagcatgcagccatctggagggagggcccagagctcatggctgccgccactggagacaagagggcggagcactcagggaggcagcccacggtctatggactgggttgtgggttgtggactgtgggctgtagggtgtggactgtgggctttgaggtgtggcctgtggtctgtgatctgtggcctgtaggctgtggcctgtggaccgtgggctgtggacagcagcctgtggactgtgggctgtggactgtggggtgtgggctgtggccttggacaagttgctgcacatccccatcatgagtacccatggcaatgaggagtacccatggcgatgaggacccatggcaatgaggagtacccatggcaatgaggagtacccatggcgatgaggacccatggcgatgaggagtacccatggcgatgaggacccatggcgatgaggagtacccatggcgatgaggacccatggcgatgaggagtacccatggcgatgaggagtacccatggcgatgaggacccatggcgatgaggagtacccatggcgatgaggagtacccatggcgatgaggacccatggcgatgaggagtacccatggcgatgaggagtacccatggcgatgaggagtacccatggcgatgagtacccattgcgatgaggagtacccatggcaatgaggagtacccatggcgatgaggagtacccatggcgatgaggagtacccatggtgatgaggacccatggcgatgaggagtacccatggcgatgagtacccatggcgatgaggagtacccatggcgatgaggagtacccatggcgatgaggagtacccatggcgatgaggacccatggcaatgaggagtacccatggcaatgaggagtacccatggcgatgaggagtacccatggcgatgaggagtacccatggcgatgaggaatacccatggcgaggagtacccatggcgatgaggagtacccatggcgatgaggagtacccatggcgaggagtacccatggcgatgaggagtacccatggcgatgaggagtacccatggcgatgaggagtacccatggcgatgaggaatacccatggcaaggagtacccatggtgatgaggagtacccatggcgatgaggagtacccatggcgaggagtacccatggcgatgaggagtacccatggtgatgaggagtacccatggcgatgaggagtacccatggcgaggagtacccatggtgatgaggagtacccatggcgatgaggagtacccatggtgatgagtacccatggccagctcatggcgtatagtggactgctgtgcctggcactcagggcaggctggagcaagtgctgtgctcatcaccatggcagcattgcagcggggcccggagggtctgtggccatcactcagagacgccccggctccgtggaacaggcacagggctggaccacggaagtgcctgagccgagacaggtgggatctgcggtttccaccctggaggggaagcttgctcacaaggagagggaagcctcagtgtgtggctgtggcctcgaacctcatccctatgaagaaggagggatgccctggagagggcggaagggccggggagggcacagcccggctggtggggtctgcagggaaccacaaaaggtggacaaggcccggcaggtgggcaagccttagccagaggtgggaggagaggagaggaccccatgccagcctgagcagcgtgggggtgcccggaggctgcagcccacactggattccatcttctctgtgaggagcagttgggaagggctcgagaggtgcttggctgcctcagagtcaggccgcggtgaagggaggcgccttttagggtgctgaggactcgagctgagactgtgggacgaggcagagaactcagcttcagcaaactagacatatgtgagcctggtgtggcttccaggcacgaacctagagtaggggtgtttgtgagtgtgaaagcactgagcctagagatctgccttgacgttagcaagacaccaacagatgtgcgagcgaggctccaggctccatcgctccctgatccgctggcggagccagaacacagagcgtggagtggaaagtgtgttttgaatttagtaaagtgttgggaagcagccactcagatactctcgtggacagagctgatggctggacacacatgtgatctgctttccctcctgaagtcccgggacaggggcagtgaagggatctcgctaaaagtacaaacccacgtgctcaaaggagggtgtgagcggcagcgtcatggcagctggaagactgatgatgggtgaggggagccggcagctgacacaaggaagcagaatgctaagctgctgccagagccctgaagctgcacagaactgtcagtgcccagtgcctggtgtccgtgcaaaggtgaccttggcagatgaatgactgcatgagagcagctgcacacagagctgtccctccgccctctgtcctgtgacggtccccacagctgtgcccagacccgtccctccatctgagacagtccctgcggctgtgcccagacccacccctccatcccgagacagttgccacggctgagcccagacccgtccttccatcccgagacagtccccatggatgcgcccagacccgtccctccatccggagacagtccccgcggctgcacccagacccatccctccatcccaagacagtccccgcggctgcgcccaaacccgcccctccatctggagacagtccccacggctgagcccagacccgtcccttcatcctgacacagtccccgtggctgcacccagacccgtccctccatcccgacacagtcccccagtccccgtggctgagcccagacccgcccctccatcccgacgcagtcccccagtccccgcggctgcacccagacccgtccctccatcccgacgcagtcccccagtccccgcggctgcacccagacccgtccctccatcccgacacagtcccccagtccccgtggctgagcccagacccgcccctccatcccgacacagtcccccagtccctgcggctgcacccagacccgtccctccatcccgacagtcccccagtccccgcagctgagcccagacccgcccctccatcccgagacagtccccgcggctgagcccagacctgcccctctatcctgacacagtctctgcagctgagaccagacccatcatcccatcctgaggcagtctccgcggctgcacccagagccgtccctccatcccgagacagtccccggggctgagcccagagccatccccccatcccgtgacagcctctgcggctgcgcccagagccctccctccatcctgagtccccgtggctgcgcccagagccgtccctccatcctgccacagtcctgtggttaagggccttcttggcagaagactgggaccggaccacctctctggagaggacacagccatagcactcctgggtcaccggacaactggagaacaggccgacagctgaggaaaaggagagtgaccgttggttgaggctccccaggcctcctctccaacgtggttcccagaatgtggaagacccgccttggcatgatctgaccagctcaagaggaaaattcaaaagagaatgatgttggattctccccagtaaaagagtccaggaaggctgcctcagtgcagctacagtcaacaagtcccgccctgtgcccagcactagagtgggcatggggcatttttggttgtcatttttggttgtcacagcctgggggtgctgctgtcaccccacaggcagagtctggggtgctgcttggcacccagtaacacacagggcagcccctccacaaaggattttctggccccaaatgtggagagtgctgaggccccgggggggatgcatccccagagcatcagtcctgcgattcctggagtgcgtgcccaccatggaggtgaccacctctgaacccgcaatgtcccttgctggcag

SEQ ID NO: 40 - DNA, 1039 bp, synthetic construct
  source 1..1039: mol_type = other DNA
tccaggggcgtgcacagggcggggccggtcatgcgcggttccaggggcgtgcacagggcggggccggtcatgcgcggtaagaggtcgacgtcccagggtctgaggagagggagcgcaggcccccatttgtaggagtgagtcagctgacccgcccccggggttcctaatctcactaagaaagactttgctgatgacagggtttcagttcagtaaggtagagctttggccgaggacgaggggaagatgggagtcaaagttctgtttgccctgatctgcatcgctgtggccgaggccaagcccaccgagaacaacgaagacttcaacatcgtggccgtggccagcaacttcgcgaccacggatctcgatgctgaccgcgggaagttgcccggcaagaagctgccgctggaggtgctcaaagagctggaagccaatgcccggaaagctggctgcaccaggggctgtctgatctgcctgtcccacatcaagtgcacgcccaagatgaagaagttcatcccaggacgctgccacacctacgaaggcgacaaagagtccgcacagggcggcataggcgaggcgatcgtcgacattcctgagattcctgggttcaaggacttggagcccctggagcagttcatcgcacaggtcgatctgtgtgtggactgcacaactggctgcctcaaagggcttgccaacgtgcagtgttctgacctgctcaagaagtggctgccgcaacgctgtgcgacctttgccagcaagatccagggccaggtggacaagatcaagggggccggtggtgactaagcggccgctcgagctgtgccttctagttgccagccatctgttgtttgcccctcccccgtgccttccttgaccctggaaggtgccactcccactgtcctttcctaataaaatgaggaaattgcatcgcattgtctgagtaggtgtcattctattctggggggtggggtggggcaggacagcaagggggaggattgggaagacaatagcaggcatgctggggatgcggtgggctctatgg

SEQ ID NO: 41 - DNA, 558 bp, synthetic construct
  source 1..558: mol_type = other DNA
atgggagtcaaagttctgtttgccctgatctgcatcgctgtggccgaggccaagcccaccgagaacaacgaagacttcaacatcgtggccgtggccagcaacttcgcgaccacggatctcgatgctgaccgcgggaagttgcccggcaagaagctgccgctggaggtgctcaaagagctggaagccaatgcccggaaagctggctgcaccaggggctgtctgatctgcctgtcccacatcaagtgcacgcccaagatgaagaagttcatcccaggacgctgccacacctacgaaggcgacaaagagtccgcacagggcggcataggcgaggcgatcgtcgacattcctgagattcctgggttcaaggacttggagcccctggagcagttcatcgcacaggtcgatctgtgtgtggactgcacaactggctgcctcaaagggcttgccaacgtgcagtgttctgacctgctcaagaagtggctgccgcaacgctgtgcgacctttgccagcaagatccagggccaggtggacaagatcaagggggccggtggtgactaa